European Patent Application EP 4 715 044 A1, published March 25, 2026. Title: 细胞治疗产品制备工艺及其应用. Applicant: 重庆精准生物技术有限公司. The sequence listing filed with the application follows.

SEQUENCE LISTING (3 sequences)

SEQ ID NO: 1 - protein, 468 aa, synthetic construct
DIQMTQSPSSLSASVGDRVTITCRASQDISKYLNWYQQKPGKAPRLLIYHTSRLHSGVPSRFSGSGSGTDYTLTISSLQPEDFATYYCQQGNTLPYTFGGGTRLEIKGSTSGSGKPGSGEGSTKGQVQLQESGPGLVKPSQTLSLTCTVSGVSLPDYGVSWIRQPPGKALEWLGVIWGSETTYYSTSLKTRLTISKDNSKNQVVLTMTNMDPVDTATYYCAKHYYYGGSYAMDYWGQGSSVTVSSTTTPAPRPPTPAPTIASQPLSLRPEACRPAAGGAVHTRGLDFACDIYIWAPLAGTCGVLLLSLVITLYCKRGRKKLLYIFKQPFMRPVQTTQEEDGCSCRFPEEEEGGCELRVKFSRSADAPAYKQGQNQLYNELNLGRREEYDVLDKRRGRDPEMGGKPRRKNPQEGLYNELQKDKMAEAYSEIGMKGERRRGKGHDGLYQGLSTATKDTYDALHMQALPPR

SEQ ID NO: 2 - protein, 965 aa, synthetic construct
DIQMTQSPSSLSASVGDRVTITCRASQDISKYLNWYQQKPGKAPRLLIYHTSRLHSGVPSRFSGSGSGTDYTLTISSLQPEDFATYYCQQGNTLPYTFGGGTRLEIKGSTSGSGKPGSGEGSTKGQVQLQESGPGLVKPSQTLSLTCTVSGVSLPDYGVSWIRQPPGKALEWLGVIWGSETTYYSTSLKTRLTISKDNSKNQVVLTMTNMDPVDTATYYCAKHYYYGGSYAMDYWGQGSSVTVSSTTTPAPRPPTPAPTIASQPLSLRPEACRPAAGGAVHTRGLDFACDIYIWAPLAGTCGVLLLSLVITLYCKRGRKKLLYIFKQPFMRPVQTTQEEDGCSCRFPEEEEGGCELRVKFSRSADAPAYKQGQNQLYNELNLGRREEYDVLDKRRGRDPEMGGKPRRKNPQEGLYNELQKDKMAEAYSEIGMKGERRRGKGHDGLYQGLSTATKDTYDALHMQALPPRGSGATNFSLLKQAGDVEENPGPETTLTQSPATLSVSPGERATLSCRASQSVSSNLAWYQQKPGQAPRLLIYGASTRATGIPARFSGSGSGTEFTLTISSLQSEDFAIYYCQQYHSWPPLTFGGGTKLEIKRGSTSGSGKPGSGEGSTKGQVQLVQSGAEVKKPGASVKVSCKASGYTFTSYGISWVRQAPGQGLEWVGWISAYNGNTIYAQKLQGRVTMTTDTSTSTAYMELRSLRSDDTAVYYCARDFQGIAVADLDYWGQGTLVTVSSKPTTTPAPRPPTPAPTIASQPLSLRPEACRPAAGGAVHTRGLDFACDFWVLVVVGGVLACYSLLVTVAFIIFWVRSKRSRGGHSDYMNMTPRRPGPTRKHYQPYAPPRDFAAYRSRVKFSRSADAPAYKQGQNQLYNELNLGRREEYDVLDKRRGRDPEMGGKPRRKNPQEGLYNELQKDKMAEAYSEIGMKGERRRGKGHDGLYQGLSTATKDTYDALHMQALPPR

SEQ ID NO: 3 - protein, 466 aa, synthetic construct
DIQMTQSPSSLSASVGDRVTITCSTSSSVSYMHWYQQKPGKAPRLLIYSTSNLASGVPSRFSGSGSGTDFTFTISSLQPEDIATYYCHQWSSYPTFGQGTKVEIKGSTSGSGKPGSGEGSTKGQVQLQESGPGLVRPSQTLSLTCTVSGFTISSGYSWHWVRQPPGRGLEWIGYIQYSGITNYNPSLKSRVTMLVDTSKNQFSLRLSSVTAADTAVYYCAREDYDYHWYFDVWGQGSTVTVSSTTTPAPRPPTPAPTIASQPLSLRPEACRPAAGGAVHTRGLDFACDIYIWAPLAGTCGVLLLSLVITLYCKRGRKKLLYIFKQPFMRPVQTTQEEDGCSCRFPEEEEGGCELRVKFSRSADAPAYKQGQNQLYNELNLGRREEYDVLDKRRGRDPEMGGKPRRKNPQEGLYNELQKDKMAEAYSEIGMKGERRRGKGHDGLYQGLSTATKDTYDALHMQALPPR